European Patent Specification EP 3 574 000 B1, published August 14, 2024. Title: HEPATITIS E VIRUS ORF2 CAPSID POLYPEPTIDES AND USES THEREOF. Applicant: Inserm. The sequence listing filed with the application follows.

SEQUENCE LISTING (3 sequences)

SEQ ID NO: 1 - protein, 647 aa, Hepatitis E virus
LPMLPAPPAGQPSGRRRGRRSGGAGGGFWGDRVDSQPFALPYIHPTNPFAADIVSQSGAGTRPRQPPRPLGSAWRDQSQRPSAAPRRRSAPAGAAPLTAVSPAPDTAPVPDVDSRGAILRRQYNLSTSPLTSSVASGTNLVLYAAPLNPLLPLQDGTNTHIMATEASNYAQYRVVRATIRYRPLVPNAVGGYAISISFWPQTTTTPTSVDMNSITSTDVRILVQPGIASELVIPSERLHYRNQGWRSVETTGVAEEEATSGLVMLCIHGSPVNSYTNTPYTGALGLLDFALELEFRNLTPGNTNTRVSRYTSTARHRLRRGADGTAELTTTAATRFMKDLHFTGTNGVGEVGRGIALTLFNLADTLLGGLPTELISSAGGQLFYSRPVVSANGEPTVKLYTSVENAQQDKGITIPHDIDLGDSRVVIQDYDNQHEQDRPTPSPAPSRPFSVLRANDVLWLSLTAAEYDQATYGSSTNPMYVSDTVTFVNVATGAQAVARSLDWSKVTLDGRPLTTIQQYSKTFYVLPLRGKLSFWEAGTTRAGYPYNYNTTASDQILIENAAGHRVAISTYTTSLGAGPASISAVGVLAPHSALAVLEDTVDYPARAHTFDDFCPECRTLGLQGCAFQSTIAELQRLKTEVGKTRES

SEQ ID NO: 2 - protein, 627 aa, Hepatitis E virus
SGGAGGGFWGDRVDSQPFALPYIHPTNPFAADIVSQSGAGTRPRQPPRPLGSAWRDQSQRPSAAPRRRSAPAGAAPLTAVSPAPDTAPVPDVDSRGAILRRQYNLSTSPLTSSVASGTNLVLYAAPLNPLLPLQDGTNTHIMATEASNYAQYRVVRATIRYRPLVPNAVGGYAISISFWPQTTTTPTSVDMNSITSTDVRILVQPGIASELVIPSERLHYRNQGWRSVETTGVAEEEATSGLVMLCIHGSPVNSYTNTPYTGALGLLDFALELEFRNLTPGNTNTRVSRYTSTARHRLRRGADGTAELTTTAATRFMKDLHFTGTNGVGEVGRGIALTLFNLADTLLGGLPTELISSAGGQLFYSRPVVSANGEPTVKLYTSVENAQQDKGITIPHDIDLGDSRVVIQDYDNQHEQDRPTPSPAPSRPFSVLRANDVLWLSLTAAEYDQATYGSSTNPMYVSDTVTFVNVATGAQAVARSLDWSKVTLDGRPLTTIQQYSKTFYVLPLRGKLSFWEAGTTRAGYPYNYNTTASDQILIENAAGHRVAISTYTTSLGAGPASISAVGVLAPHSALAVLEDTVDYPARAHTFDDFCPECRTLGLQGCAFQSTIAELQRLKTEVGKTRES

SEQ ID NO: 3 - protein, 660 aa, Hepatitis E virus
MCPRVVLLLFFVFLPMLPAPPAGQPSGRRRGRRSGGAGGGFWGDRVDSQPFALPYIHPTNPFAADIVSQSGAGTRPRQPPRPLGSAWRDQSQRPSAAPRRRSAPAGAAPLTAVSPAPDTAPVPDVDSRGAILRRQYNLSTSPLTSSVASGTNLVLYAAPLNPLLPLQDGTNTHIMATEASNYAQYRVVRATIRYRPLVPNAVGGYAISISFWPQTTTTPTSVDMNSITSTDVRILVQPGIASELVIPSERLHYRNQGWRSVETTGVAEEEATSGLVMLCIHGSPVNSYTNTPYTGALGLLDFALELEFRNLTPGNTNTRVSRYTSTARHRLRRGADGTAELTTTAATRFMKDLHFTGTNGVGEVGRGIALTLFNLADTLLGGLPTELISSAGGQLFYSRPVVSANGEPTVKLYTSVENAQQDKGITIPHDIDLGDSRVVIQDYDNQHEQDRPTPSPAPSRPFSVLRANDVLWLSLTAAEYDQATYGSSTNPMYVSDTVTFVNVATGAQAVARSLDWSKVTLDGRPLTTIQQYSKTFYVLPLRGKLSFWEAGTTRAGYPYNYNTTASDQILIENAAGHRVAISTYTTSLGAGPASISAVGVLAPHSALAVLEDTVDYPARAHTFDDFCPECRTLGLQGCAFQSTIAELQRLKTEVGKTRES